European Patent Application EP 4 711 456 A1, published March 18, 2026. Title: Method for the manufacture of individualized CRISPR/Cas complexes and individualized CRISPR/Cas complexes. Applicant: GenCC GmbH & Co. KG. Application EP. The sequence listing filed with the application follows.

SEQUENCE LISTING (96 sequences)

SEQ ID NO: 1 - protein, 296 aa, Homo sapiens
MAAGGPGAGSAAPVSSTSSLPLAALNMRVRRRLSLFLNVRTQVAADWTALAEEMDFEYLEIRQLETQADPTGRLLDAWQGRPGASVGRLLELLTKLGRDDVLLELGPSIEEDCQKYILKQQQEEAEKPLQVAAVDSSVPRTAELAGITTLDDPLGHMPERFDAFICYCPSDIQFVQEMIRQLEQTNYRLKLCVSDRDVLPGTCVWSIASELIEKRCRRMVVVVSDDYLQSKECDFQTKFALSLSPGAHQKRLIPIKYKAMKKEFPSILRFITVCDYTNPCTKSWFWTRLAKALSLP

SEQ ID NO: 2 - DNA, 65 bp, Homo sapiens
  source 1..65: mol_type = genomic DNA
cccttggcttgcaggtgcccatcagaagcgactgatccccatcaagtacaaggcaatgaagaaag

SEQ ID NO: 3 - RNA, 20 nt, synthetic construct
  source 1..20: mol_type = other RNA
gccttgtacttgatggggat

SEQ ID NO: 4 - RNA, 20 nt, synthetic construct
  source 1..20: mol_type = other RNA
ggggatcggtcgcttctgat

SEQ ID NO: 5 - RNA, 16 nt, synthetic construct
  source 1..16: mol_type = other RNA
gttttagagctatgct

SEQ ID NO: 6 - RNA, 36 nt, synthetic construct
  source 1..36: mol_type = other RNA
gccttgtacttgatggggatgttttagagctatgct

SEQ ID NO: 7 - RNA, 36 nt, synthetic construct
  source 1..36: mol_type = other RNA
ggggatcggtcgcttctgatgttttagagctatgct

SEQ ID NO: 8 - RNA, 36 nt, synthetic construct
  source 1..36: mol_type = other RNA
gtacttggagatccggcaacgttttagagctatgct

SEQ ID NO: 9 - RNA, 36 nt, synthetic construct
  source 1..36: mol_type = other RNA
atgaaggcatcgaaacgctcgttttagagctatgct

SEQ ID NO: 10 - DNA, 20 bp, synthetic construct
  source 1..20: mol_type = other DNA
tggattgtcagccttccctc

SEQ ID NO: 11 - DNA, 20 bp, synthetic construct
  source 1..20: mol_type = other DNA
gccttgtacttgatggggat

SEQ ID NO: 12 - DNA, 20 bp, synthetic construct
  source 1..20: mol_type = other DNA
ctcaagggtagaggtgggca

SEQ ID NO: 13 - DNA, 19 bp, synthetic construct
  source 1..19: mol_type = other DNA
ggggacgtcctcaccaatg

SEQ ID NO: 14 - DNA, 20 bp, synthetic construct
  source 1..20: mol_type = other DNA
tcatcttgggaagggtgcag

SEQ ID NO: 15 - DNA, 20 bp, synthetic construct
  source 1..20: mol_type = other DNA
gcaggtcctgtggcaactta

SEQ ID NO: 16 - RNA, 20 nt, synthetic construct
  source 1..20: mol_type = other RNA
ggggatcggtcgcttctgat

SEQ ID NO: 17 - RNA, 20 nt, synthetic construct
  source 1..20: mol_type = other RNA
tggggatcggtcgcttctga

SEQ ID NO: 18 - RNA, 20 nt, synthetic construct
  source 1..20: mol_type = other RNA
accgatccccatcaagtaca

SEQ ID NO: 19 - RNA, 25 nt, synthetic construct
  source 1..25: mol_type = other RNA
attgccttgtacttgatggggatca

SEQ ID NO: 20 - RNA, 23 nt, synthetic construct
  source 1..23: mol_type = other RNA
tgatggggatcggtcgcttctga

SEQ ID NO: 21 - RNA, 23 nt, synthetic construct
  source 1..23: mol_type = other RNA
catcagaagcgaccgatccccat

SEQ ID NO: 22 - RNA, 22 nt, synthetic construct
  source 1..22: mol_type = other RNA
tgatggggatcggtcgcttctg

SEQ ID NO: 23 - RNA, 22 nt, synthetic construct
  source 1..22: mol_type = other RNA
catcagaagcgaccgatcccca

SEQ ID NO: 24 - RNA, 26 nt, synthetic construct
  source 1..26: mol_type = other RNA
ttncaggtgcccatcagaagcgaccg

SEQ ID NO: 25 - RNA, 26 nt, synthetic construct
  source 1..26: mol_type = other RNA
ttnatggggatcggtcgcttctgatg

SEQ ID NO: 26 - RNA, 26 nt, synthetic construct
  source 1..26: mol_type = other RNA
ttntacttgatggggatcggtcgctt

SEQ ID NO: 27 - RNA, 26 nt, synthetic construct
  source 1..26: mol_type = other RNA
ttnccttgtacttgatggggatcggt

SEQ ID NO: 28 - RNA, 20 nt, synthetic construct
  source 1..20: mol_type = other RNA
gcaggtgcccatcagaagcg

SEQ ID NO: 29 - RNA, 20 nt, synthetic construct
  source 1..20: mol_type = other RNA
cttgatggggatcggtcgct

SEQ ID NO: 30 - RNA, 20 nt, synthetic construct
  source 1..20: mol_type = other RNA
tcagaagcgaccgatcccca

SEQ ID NO: 31 - RNA, 20 nt, synthetic construct
  source 1..20: mol_type = other RNA
ttgccttgtacttgatgggg

SEQ ID NO: 32 - RNA, 20 nt, synthetic construct
  source 1..20: mol_type = other RNA
ccgatccccatcaagtacaa

SEQ ID NO: 33 - RNA, 20 nt, synthetic construct
  source 1..20: mol_type = other RNA
aggtgcccatcagaagcgac

SEQ ID NO: 34 - RNA, 20 nt, synthetic construct
  source 1..20: mol_type = other RNA
tgatggggatcggtcgcttc

SEQ ID NO: 35 - RNA, 20 nt, synthetic construct
  source 1..20: mol_type = other RNA
gaagcgaccgatccccatca

SEQ ID NO: 36 - RNA, 20 nt, synthetic construct
  source 1..20: mol_type = other RNA
ccttgtacttgatggggatc

SEQ ID NO: 37 - RNA, 23 nt, synthetic construct
  source 1..23: mol_type = other RNA
caggtgcccatcagaagcgaccg

SEQ ID NO: 38 - RNA, 23 nt, synthetic construct
  source 1..23: mol_type = other RNA
atggggatcggtcgcttctgatg

SEQ ID NO: 39 - RNA, 23 nt, synthetic construct
  source 1..23: mol_type = other RNA
tacttgatggggatcggtcgctt

SEQ ID NO: 40 - RNA, 23 nt, synthetic construct
  source 1..23: mol_type = other RNA
ccttgtacttgatggggatcggt

SEQ ID NO: 41 - RNA, 23 nt, synthetic construct
  source 1..23: mol_type = other RNA
ccttgtacttgatggggatcggt

SEQ ID NO: 42 - RNA, 23 nt, synthetic construct
  source 1..23: mol_type = other RNA
ccttgtacttgatggggatcggt

SEQ ID NO: 43 - RNA, 23 nt, synthetic construct
  source 1..23: mol_type = other RNA
ccttgtacttgatggggatcggt

SEQ ID NO: 44 - RNA, 20 nt, synthetic construct
  source 1..20: mol_type = other RNA
ggtgcccatcagaagcgacc

SEQ ID NO: 45 - RNA, 20 nt, synthetic construct
  source 1..20: mol_type = other RNA
gggatcggtcgcttctgatg

SEQ ID NO: 46 - RNA, 20 nt, synthetic construct
  source 1..20: mol_type = other RNA
gtgcccatcagaagcgaccg

SEQ ID NO: 47 - RNA, 24 nt, synthetic construct
  source 1..24: mol_type = other RNA
ttgccttgtacttgatggggatcg

SEQ ID NO: 48 - RNA, 20 nt, synthetic construct
  source 1..20: mol_type = other RNA
atcggtcgcttctgatgggc

SEQ ID NO: 49 - RNA, 20 nt, synthetic construct
  source 1..20: mol_type = other RNA
atggggatcggtcgcttctg

SEQ ID NO: 50 - RNA, 20 nt, synthetic construct
  source 1..20: mol_type = other RNA
tcagaagcgaccgatcccca

SEQ ID NO: 51 - RNA, 20 nt, synthetic construct
  source 1..20: mol_type = other RNA
cgaccgatccccatcaagta

SEQ ID NO: 52 - RNA, 23 nt, synthetic construct
  source 1..23: mol_type = other RNA
cccatcagaagcgaccgatcccc

SEQ ID NO: 53 - RNA, 23 nt, synthetic construct
  source 1..23: mol_type = other RNA
cttgatggggatcggtcgcttct

SEQ ID NO: 54 - RNA, 20 nt, synthetic construct
  source 1..20: mol_type = other RNA
tcggtcgcttctgatgggca

SEQ ID NO: 55 - RNA, 20 nt, synthetic construct
  source 1..20: mol_type = other RNA
ggatcggtcgcttctgatgg

SEQ ID NO: 56 - RNA, 20 nt, synthetic construct
  source 1..20: mol_type = other RNA
gtgcccatcagaagcgaccg

SEQ ID NO: 57 - RNA, 20 nt, synthetic construct
  source 1..20: mol_type = other RNA
ccatcagaagcgaccgatcc

SEQ ID NO: 58 - RNA, 20 nt, synthetic construct
  source 1..20: mol_type = other RNA
gtacttgatggggatcggtc

SEQ ID NO: 59 - RNA, 20 nt, synthetic construct
  source 1..20: mol_type = other RNA
gaagcgaccgatccccatca

SEQ ID NO: 60 - RNA, 20 nt, synthetic construct
  source 1..20: mol_type = other RNA
gaccgatccccatcaagtac

SEQ ID NO: 61 - RNA, 20 nt, synthetic construct
  source 1..20: mol_type = other RNA
cattgccttgtacttgatgg

SEQ ID NO: 62 - RNA, 20 nt, synthetic construct
  source 1..20: mol_type = other RNA
atggggatcggtcgcttctg

SEQ ID NO: 63 - RNA, 20 nt, synthetic construct
  source 1..20: mol_type = other RNA
tacttgatggggatcggtcg

SEQ ID NO: 64 - RNA, 20 nt, synthetic construct
  source 1..20: mol_type = other RNA
ggtgcccatcagaagcgacc

SEQ ID NO: 65 - RNA, 20 nt, synthetic construct
  source 1..20: mol_type = other RNA
catcagaagcgaccgatccc

SEQ ID NO: 66 - RNA, 20 nt, synthetic construct
  source 1..20: mol_type = other RNA
gaagcgaccgatccccatca

SEQ ID NO: 67 - RNA, 20 nt, synthetic construct
  source 1..20: mol_type = other RNA
ccttgtacttgatggggatc

SEQ ID NO: 68 - RNA, 20 nt, synthetic construct
  source 1..20: mol_type = other RNA
tggggatcggtcgcttctga

SEQ ID NO: 69 - RNA, 20 nt, synthetic construct
  source 1..20: mol_type = other RNA
atggggatcggtcgcttctg

SEQ ID NO: 70 - RNA, 20 nt, synthetic construct
  source 1..20: mol_type = other RNA
gaccgatccccatcaagtac

SEQ ID NO: 71 - RNA, 22 nt, synthetic construct
  source 1..22: mol_type = other RNA
cagaagcgaccgatccccatca

SEQ ID NO: 72 - RNA, 20 nt, synthetic construct
  source 1..20: mol_type = other RNA
tggggatcggtcgcttctga

SEQ ID NO: 73 - RNA, 20 nt, synthetic construct
  source 1..20: mol_type = other RNA
ggtcgcttctgatgggcacc

SEQ ID NO: 74 - RNA, 20 nt, synthetic construct
  source 1..20: mol_type = other RNA
aggtgcccatcagaagcgac

SEQ ID NO: 75 - RNA, 20 nt, synthetic construct
  source 1..20: mol_type = other RNA
ggtgcccatcagaagcgacc

SEQ ID NO: 76 - RNA, 20 nt, synthetic construct
  source 1..20: mol_type = other RNA
gatcggtcgcttctgatggg

SEQ ID NO: 77 - RNA, 20 nt, synthetic construct
  source 1..20: mol_type = other RNA
gggatcggtcgcttctgatg

SEQ ID NO: 78 - RNA, 20 nt, synthetic construct
  source 1..20: mol_type = other RNA
ggggatcggtcgcttctgat

SEQ ID NO: 79 - RNA, 20 nt, synthetic construct
  source 1..20: mol_type = other RNA
catcagaagcgaccgatccc

SEQ ID NO: 80 - RNA, 20 nt, synthetic construct
  source 1..20: mol_type = other RNA
tgatggggatcggtcgcttc

SEQ ID NO: 81 - RNA, 20 nt, synthetic construct
  source 1..20: mol_type = other RNA
agaagcgaccgatccccatc

SEQ ID NO: 82 - RNA, 20 nt, synthetic construct
  source 1..20: mol_type = other RNA
gaagcgaccgatccccatca

SEQ ID NO: 83 - RNA, 20 nt, synthetic construct
  source 1..20: mol_type = other RNA
agcgaccgatccccatcaag

SEQ ID NO: 84 - RNA, 20 nt, synthetic construct
  source 1..20: mol_type = other RNA
tgtacttgatggggatcggt

SEQ ID NO: 85 - RNA, 20 nt, synthetic construct
  source 1..20: mol_type = other RNA
ccttgtacttgatggggatc

SEQ ID NO: 86 - RNA, 20 nt, synthetic construct
  source 1..20: mol_type = other RNA
accgatccccatcaagtaca

SEQ ID NO: 87 - RNA, 20 nt, synthetic construct
  source 1..20: mol_type = other RNA
gccttgtacttgatggggat

SEQ ID NO: 88 - RNA, 20 nt, synthetic construct
  source 1..20: mol_type = other RNA
ccgatccccatcaagtacaa

SEQ ID NO: 89 - RNA, 20 nt, synthetic construct
  source 1..20: mol_type = other RNA
tggggatcggtcgcttctga

SEQ ID NO: 90 - RNA, 20 nt, synthetic construct
  source 1..20: mol_type = other RNA
tgcaggtgcccatcagaagc

SEQ ID NO: 91 - RNA, 20 nt, synthetic construct
  source 1..20: mol_type = other RNA
ggtcgcttctgatgggcacc

SEQ ID NO: 92 - RNA, 20 nt, synthetic construct
  source 1..20: mol_type = other RNA
gatcggtcgcttctgatggg

SEQ ID NO: 93 - RNA, 20 nt, synthetic construct
  source 1..20: mol_type = other RNA
gggatcggtcgcttctgatg

SEQ ID NO: 94 - RNA, 20 nt, synthetic construct
  source 1..20: mol_type = other RNA
agcgaccgatccccatcaag

SEQ ID NO: 95 - RNA, 20 nt, synthetic construct
  source 1..20: mol_type = other RNA
tgtacttgatggggatcggt

SEQ ID NO: 96 - RNA, 20 nt, synthetic construct
  source 1..20: mol_type = other RNA
ccgatccccatcaagtacaa